European Patent Application EP 4 219 725 A2, published August 2, 2023. Title: ALTERING GENE EXPRESSION IN MODIFIED T CELLS AND USES THEREOF. Applicant: The Trustees of the University of Pennsylvania. Application EP. The sequence listing filed with the application follows.

SEQUENCE LISTING (68 sequences)

SEQ ID NO: 1 - DNA, 20 bp, synthetic construct
  misc_feature 1..20: note = Synthetic sequence
  source 1..20: mol_type = other DNA
tgtgctagacatgaggtcta

SEQ ID NO: 2 - DNA, 20 bp, synthetic construct
  misc_feature 1..20: note = Synthetic sequence
  source 1..20: mol_type = other DNA
gcagtatctggagtcattga

SEQ ID NO: 3 - DNA, 20 bp, synthetic construct
  misc_feature 1..20: note = Synthetic sequence
  source 1..20: mol_type = other DNA
cgcgagcacagctaaggcca

SEQ ID NO: 4 - DNA, 20 bp, synthetic construct
  misc_feature 1..20: note = Synthetic sequence
  source 1..20: mol_type = other DNA
ggcgccctggccagtcgtct

SEQ ID NO: 5 - DNA, 20 bp, synthetic construct
  misc_feature 1..20: note = Synthetic sequence
  source 1..20: mol_type = other DNA
gagggtccagatgcccagca

SEQ ID NO: 6 - DNA, 24 bp, synthetic construct
  misc_feature 1..24: note = Synthetic sequence
  source 1..24: mol_type = other DNA
tcatgtcctaaccctgatcctctt

SEQ ID NO: 7 - DNA, 23 bp, synthetic construct
  misc_feature 1..23: note = Synthetic sequence
  source 1..23: mol_type = other DNA
ttggacttttcccagctgacaga

SEQ ID NO: 8 - DNA, 24 bp, synthetic construct
  misc_feature 1..24: note = Synthetic sequence
  source 1..24: mol_type = other DNA
taccaggaccagacagctcttaga

SEQ ID NO: 9 - DNA, 24 bp, synthetic construct
  misc_feature 1..24: note = Synthetic sequence
  source 1..24: mol_type = other DNA
tctcacctaatctcctccaggcat

SEQ ID NO: 10 - RNA, 27 nt, synthetic construct
  misc_feature 1..27: note = Synthetic sequence
  source 1..27: mol_type = other RNA
  misc_feature 1..27: note = siRNA
aggaggattcggaacccaatcactgac

SEQ ID NO: 11 - DNA, 25 bp, synthetic construct
  misc_feature 1..25: note = Synthetic sequence
  source 1..25: mol_type = other DNA
  misc_feature 1..23: note = RNA
  misc_feature 24..25: note = DNA
  misc_feature 1..25: note = siRNA
cagtgattgggttccgaatcctcct

SEQ ID NO: 12 - RNA, 27 nt, synthetic construct
  misc_feature 1..27: note = Synthetic sequence
  source 1..27: mol_type = other RNA
  misc_feature 1..27: note = siRNA
acctccttcccattcacccaccagctc

SEQ ID NO: 13 - DNA, 25 bp, synthetic construct
  misc_feature 1..25: note = Synthetic sequence
  source 1..25: mol_type = other DNA
  misc_feature 1..23: note = RNA
  misc_feature 24..25: note = DNA
  misc_feature 1..25: note = siRNA
gctggtgggtgaatgggaaggaggt

SEQ ID NO: 14 - DNA, 122 bp, synthetic construct
  misc_feature 1..122: note = Synthetic sequence; Figure 1B
  source 1..122: mol_type = other DNA
ttaatacgactcactataggcaccaaagctgcccttaccgttttagagctagaaatagcaagttaaaataaggctagtccgttatcaacttgaaaaagtggcaccgagtcggtgcttttttt

SEQ ID NO: 15 - DNA, 23 bp, synthetic construct
  misc_feature 1..23: note = Synthetic sequence; Figure 1C, Figure 3B, & Figure 21
  source 1..23: mol_type = other DNA
tgtgctagacatgaggtctatgg

SEQ ID NO: 16 - DNA, 23 bp, synthetic construct
  misc_feature 1..23: note = Synthetic sequence; Figure 1C, Figure 3B, & Figure 21
  source 1..23: mol_type = other DNA
ccctcaatgactccagatactgc

SEQ ID NO: 17 - DNA, 38 bp, synthetic construct
  misc_feature 1..38: note = Synthetic sequence; Figure 79B
  source 1..38: mol_type = other DNA
tgggctggcggccaggatggttcttggtaggtaggtgg

SEQ ID NO: 18 - DNA, 38 bp, synthetic construct
  misc_feature 1..38: note = Synthetic sequence; Figure 79B
  source 1..38: mol_type = other DNA
tgggctggcggccaggatggttcttaggggtaggtggg

SEQ ID NO: 19 - DNA, 67 bp, synthetic construct
  misc_feature 1..67: note = Synthetic sequence; Figure 3D & Figure 53A
  source 1..67: mol_type = other DNA
tatatcacagacaaaactgtgctagacatgaggtctatggacttcaagagcaacagtgctgtggcct

SEQ ID NO: 20 - DNA, 66 bp, synthetic construct
  misc_feature 1..66: note = Synthetic sequence; Figure 3D & Figure 53A
  source 1..66: mol_type = other DNA
tatatcacagacaaaactgtgctagacatgagtctatggacttcaagagcaacagtgctgtggcct

SEQ ID NO: 21 - DNA, 65 bp, synthetic construct
  misc_feature 1..65: note = Synthetic sequence; Figure 3D & Figure 53A
  source 1..65: mol_type = other DNA
tatatcacagacaaaactgtgctagacatggtctatggacttcaagagcaacagtgctgtggcct

SEQ ID NO: 22 - DNA, 66 bp, synthetic construct; identical to SEQ ID NO: 20
  misc_feature 1..66: note = Synthetic sequence; Figure 3D & Figure 53A
  source 1..66: mol_type = other DNA

SEQ ID NO: 23 - DNA, 64 bp, synthetic construct
  misc_feature 1..64: note = Synthetic sequence; Figure 3D & Figure 53A
  source 1..64: mol_type = other DNA
tatatcacagacaaaactgtgctagacatgtctatggacttcaagagcaacagtgctgtggcct

SEQ ID NO: 24 - DNA, 66 bp, synthetic construct
  misc_feature 1..66: note = Synthetic sequence; Figure 3D & Figure 53A
  source 1..66: mol_type = other DNA
tatatcacagacaaaactgtgctagactgaggtctatggacttcaagagcaacagtgctgtggcct

SEQ ID NO: 25 - DNA, 64 bp, synthetic construct
  misc_feature 1..64: note = Synthetic sequence; Figure 3D & Figure 53A
  source 1..64: mol_type = other DNA
tatatcacagacaaaactgtgctagtgaggtctatggacttcaagagcaacagtgctgtggcct

SEQ ID NO: 26 - DNA, 62 bp, synthetic construct
  misc_feature 1..62: note = Synthetic sequence; Figure 3D & Figure 53A
  source 1..62: mol_type = other DNA
tatatcacagacaaaactgtgcttgaggtctatggacttcaagagcaacagtgctgtggcct

SEQ ID NO: 27 - DNA, 67 bp, synthetic construct
  misc_feature 1..67: note = Synthetic sequence; Figure 3D & Figure 53A
  source 1..67: mol_type = other DNA
tatatcacagacaaaactgtgctagacatgaggttctatggacttcaagagcaacagtgctgtggcc

SEQ ID NO: 28 - DNA, 67 bp, synthetic construct
  misc_feature 1..67: note = Synthetic sequence; Figure 3D & Figure 53A
  source 1..67: mol_type = other DNA
tatatcacagacaaaactgtgctagacatgagggtctatggacttcaagagcaacagtgctgtggcc

SEQ ID NO: 29 - DNA, 67 bp, synthetic construct
  misc_feature 1..67: note = Synthetic sequence; Figure 3D & Figure 53A
  source 1..67: mol_type = other DNA
agcagcccgccctcaatgactccagatactgcctgagcagccgcctgagggtctcggccaccttctg

SEQ ID NO: 30 - DNA, 66 bp, synthetic construct
  misc_feature 1..66: note = Synthetic sequence; Figure 3D & Figure 53A
  source 1..66: mol_type = other DNA
agcagcccgccctcatgactccagatactgcctgagcagccgcctgagggtctcggccaccttctg

SEQ ID NO: 31 - DNA, 66 bp, synthetic construct
  misc_feature 1..66: note = Synthetic sequence; Figure 3D & Figure 53A
  source 1..66: mol_type = other DNA
agcagcccgcctcaatgactccagatactgcctgagcagccgcctgagggtctcggccaccttctg

SEQ ID NO: 32 - DNA, 66 bp, synthetic construct
  misc_feature 1..66: note = Synthetic sequence; Figure 3D & Figure 53A
  source 1..66: mol_type = other DNA
agcagcccgccctcaatgactcagatactgcctgagcagccgcctgagggtctcggccaccttctg

SEQ ID NO: 33 - DNA, 65 bp, synthetic construct
  misc_feature 1..65: note = Synthetic sequence; Figure 3D & Figure 53A
  source 1..65: mol_type = other DNA
agcagcccgccctcaatgactagatactgcctgagcagccgcctgagggtctcggccaccttctg

SEQ ID NO: 34 - DNA, 62 bp, synthetic construct
  misc_feature 1..62: note = Synthetic sequence; Figure 3D & Figure 53A
  source 1..62: mol_type = other DNA
agcagcccgcccgactccagatactgcctgagcagccgcctgagggtctcggccaccttctg

SEQ ID NO: 35 - DNA, 67 bp, synthetic construct
  misc_feature 1..67: note = Synthetic sequence; Figure 3D & Figure 53A
  source 1..67: mol_type = other DNA
agcagcccgccctcaaatgactccagatactgcctgagcagccgcctgagggtctcggccaccttct

SEQ ID NO: 36 - DNA, 67 bp, synthetic construct
  misc_feature 1..67: note = Synthetic sequence; Figure 3D & Figure 53A
  source 1..67: mol_type = other DNA
agcagcccgccctcaatgactcccagatactgcctgagcagccgcctgagggtctcggccaccttct

SEQ ID NO: 37 - DNA, 67 bp, synthetic construct; identical to SEQ ID NO: 29
  misc_feature 1..67: note = Synthetic sequence; Figure 3D & Figure 53A
  source 1..67: mol_type = other DNA

SEQ ID NO: 38 - DNA, 64 bp, synthetic construct
  misc_feature 1..64: note = Synthetic sequence; Figure 3D & Figure 53A
  source 1..64: mol_type = other DNA
agcagcccgccctcaatgacagatactgcctgagcagccgcctgagggtctcggccaccttctg

SEQ ID NO: 39 - DNA, 66 bp, synthetic construct; identical to SEQ ID NO: 32
  misc_feature 1..66: note = Synthetic sequence; Figure 3D & Figure 53A
  source 1..66: mol_type = other DNA

SEQ ID NO: 40 - DNA, 55 bp, synthetic construct
  misc_feature 1..55: note = Synthetic sequence; Figure 3D & Figure 53A
  source 1..55: mol_type = other DNA
agcagcccgccctcaactgcctgagcagccgcctgagggtctcggccaccttctg

SEQ ID NO: 41 - DNA, 62 bp, synthetic construct
  misc_feature 1..62: note = Synthetic sequence; Figure 3D & Figure 53A
  source 1..62: mol_type = other DNA
agcagcccgcctcatgactcagatactgctgagcagccgcctgagggtctcggccaccttct

SEQ ID NO: 42 - DNA, 46 bp, synthetic construct
  misc_feature 1..46: note = Synthetic sequence; Figure 3D & Figure 53A
  source 1..46: mol_type = other DNA
agcagccactgcgtgagcagccgcgtgagggtctcggccaccttct

SEQ ID NO: 43 - DNA, 67 bp, synthetic construct
  misc_feature 1..67: note = Synthetic sequence; Figure 3D & Figure 53A
  source 1..67: mol_type = other DNA
agcagcccgccctcaatgactccgagatactgcctgagcagccgcctgagggtctcggccaccttct

SEQ ID NO: 44 - DNA, 23 bp, synthetic construct
  misc_feature 1..23: note = Synthetic sequence; Figure 9A
  source 1..23: mol_type = other DNA
ccgtggccttagctgtgctcgcg

SEQ ID NO: 45 - DNA, 23 bp, synthetic construct
  misc_feature 1..23: note = Synthetic sequence; Figure 12A
  source 1..23: mol_type = other DNA
ccatgctgggcatctggaccctc

SEQ ID NO: 46 - DNA, 23 bp, synthetic construct
  misc_feature 1..23: note = Synthetic sequence; Figure 14A
  source 1..23: mol_type = other DNA
gggcggtgctacaactgggctgg

SEQ ID NO: 47 - DNA, 23 bp, synthetic construct
  misc_feature 1..23: note = Synthetic sequence; Figure 15A
  source 1..23: mol_type = other DNA
cataaagccatggcttgccttgg

SEQ ID NO: 48 - DNA, 64 bp, synthetic construct
  misc_feature 1..64: note = Synthetic sequence; Figure 15B
  source 1..64: mol_type = other DNA
aacaccgctcccataaagccatggcttgccttggatttcagcggcacaaggctcagctgaacct

SEQ ID NO: 49 - DNA, 59 bp, synthetic construct
  misc_feature 1..59: note = Synthetic sequence; Figure 15B
  source 1..59: mol_type = other DNA
aacaccgctcccataatggcttgccttggatttcagcggcacaaggctcagctgaacct

SEQ ID NO: 50 - DNA, 62 bp, synthetic construct
  misc_feature 1..62: note = Synthetic sequence; Figure 15B
  source 1..62: mol_type = other DNA
aacaccgctcccataaccatggcttgccttggatttcagcggcacaaggctcagctgaacct

SEQ ID NO: 51 - DNA, 62 bp, synthetic construct; identical to SEQ ID NO: 50
  misc_feature 1..62: note = Synthetic sequence; Figure 15B
  source 1..62: mol_type = other DNA

SEQ ID NO: 52 - DNA, 64 bp, synthetic construct
  misc_feature 1..64: note = Synthetic sequence; Figure 15B
  source 1..64: mol_type = other DNA
aacaccgctcccataaagtccatggcttgccttggatttcagcggcacaaggctcagctgaacc

SEQ ID NO: 53 - DNA, 63 bp, synthetic construct
  misc_feature 1..63: note = Synthetic sequence; Figure 15B
  source 1..63: mol_type = other DNA
aacaccgctcccataaaccatggcttgccttggatttcagcggcacaaggctcagctgaacct

SEQ ID NO: 54 - DNA, 50 bp, synthetic construct
  misc_feature 1..50: note = Synthetic sequence; Figure 15B
  source 1..50: mol_type = other DNA
aacaccgctcccataaagggatttcagcggcacaaggctcagctgaacct

SEQ ID NO: 55 - DNA, 59 bp, synthetic construct; identical to SEQ ID NO: 49
  misc_feature 1..59: note = Synthetic sequence; Figure 15B
  source 1..59: mol_type = other DNA

SEQ ID NO: 56 - DNA, 59 bp, synthetic construct; identical to SEQ ID NO: 49
  misc_feature 1..59: note = Synthetic sequence; Figure 15B
  source 1..59: mol_type = other DNA

SEQ ID NO: 57 - DNA, 63 bp, synthetic construct; identical to SEQ ID NO: 53
  misc_feature 1..63: note = Synthetic sequence; Figure 15B
  source 1..63: mol_type = other DNA

SEQ ID NO: 58 - DNA, 61 bp, synthetic construct
  misc_feature 1..61: note = Synthetic sequence; Figure 15B
  source 1..61: mol_type = other DNA
aacaccgctcccataccatggcttgccttggatttcagcggcacaaggctcagctgaacct

SEQ ID NO: 59 - DNA, 59 bp, synthetic construct; identical to SEQ ID NO: 49
  misc_feature 1..59: note = Synthetic sequence; Figure 15B
  source 1..59: mol_type = other DNA

SEQ ID NO: 60 - DNA, 64 bp, synthetic construct; identical to SEQ ID NO: 48
  misc_feature 1..64: note = Synthetic sequence; Figure 15B
  source 1..64: mol_type = other DNA

SEQ ID NO: 61 - DNA, 23 bp, synthetic construct
  misc_feature 1..23: note = Synthetic sequence; Figure 16
  source 1..23: mol_type = other DNA
ggacatcaagcctgctaacatgg

SEQ ID NO: 62 - DNA, 23 bp, synthetic construct
  misc_feature 1..23: note = Synthetic sequence; Figure 16
  source 1..23: mol_type = other DNA
catcaagcctgctaacatggagg

SEQ ID NO: 63 - DNA, 122 bp, synthetic construct
  misc_feature 1..122: note = Synthetic sequence; Figure 49
  misc_feature 19..39: note = n is a, c, g, or t
  source 1..122: mol_type = other DNA
taatacgactcactatagnnnnnnnnnnnnnnnnnnnnngttttagagctagaaatagcaagttaaaataaggctagtccgttatcaacttgaaaaagtggcaccgagtcggtgcttttttt

SEQ ID NO: 64 - DNA, 20 bp, synthetic construct
  misc_feature 1..20: note = Synthetic sequence; Figure 79A
  source 1..20: mol_type = other DNA
ggccaggatggttcttaggt

SEQ ID NO: 65 - DNA, 38 bp, synthetic construct
  misc_feature 1..38: note = Synthetic sequence; Figure 79B
  source 1..38: mol_type = other DNA
tgggctggcggccaggatggttcttaggtaggtggggt

SEQ ID NO: 66 - DNA, 34 bp, synthetic construct
  misc_feature 1..34: note = Synthetic sequence; Figure 79B
  source 1..34: mol_type = other DNA
tgggctggcggccaggatggtaggtaggtggggt

SEQ ID NO: 67 - DNA, 37 bp, synthetic construct
  misc_feature 1..37: note = Synthetic sequence; Figure 79B
  source 1..37: mol_type = other DNA
tgggctggcggccaggatggttttaggtaggtggggt

SEQ ID NO: 68 - DNA, 34 bp, synthetic construct; identical to SEQ ID NO: 66
  misc_feature 1..34: note = Synthetic sequence; Figure 79B
  source 1..34: mol_type = other DNA